European Patent Application EP 4 789 680 A1, published August 12, 2026. Title: 一种新型PACE4抑制剂及其在抗骨关节炎中的应用. Applicant: 安炎达医药技术（广州）有限公司. Application WO. The sequence listing filed with the application follows.

SEQUENCE LISTING (25 sequences)

SEQ ID NO: 1 - protein, 4 aa, synthetic construct
RFKR

SEQ ID NO: 2 - protein, 5 aa, synthetic construct
RFKRT

SEQ ID NO: 3 - protein, 5 aa, synthetic construct
  SITE 5: note = T is dT
RFKRT

SEQ ID NO: 4 - protein, 6 aa, synthetic construct
  SITE 6: note = T is dT
RRFKRT

SEQ ID NO: 5 - protein, 6 aa, synthetic construct
  SITE 1: note = R is dR
  SITE 6: note = T is dT
RRFKRT

SEQ ID NO: 6 - protein, 7 aa, synthetic construct
  SITE 2: note = R is dR
  SITE 7: note = T is dT
PRRFKRT

SEQ ID NO: 7 - protein, 7 aa, synthetic construct
  SITE 1: note = P is dP
  SITE 2: note = R is dR
  SITE 7: note = T is dT
PRRFKRT

SEQ ID NO: 8 - protein, 5 aa, synthetic construct
  SITE 2: note = F is 4-CF3 modified F
RFKRT

SEQ ID NO: 9 - protein, 5 aa, synthetic construct
  SITE 2: note = F is 4-CF3 modified F
  SITE 5: note = T is dT
RFKRT

SEQ ID NO: 10 - protein, 6 aa, synthetic construct
  SITE 3: note = F is 4-CF3 modified F
  SITE 6: note = T is dT
RRFKRT

SEQ ID NO: 11 - protein, 6 aa, synthetic construct
  SITE 1: note = R is dR
  SITE 3: note = F is 4-CF3 modified F
  SITE 6: note = T is dT
RRFKRT

SEQ ID NO: 12 - protein, 7 aa, synthetic construct
  SITE 2: note = R is dR
  SITE 4: note = F is 4-CF3 modified F
  SITE 7: note = T is dT
PRRFKRT

SEQ ID NO: 13 - protein, 7 aa, synthetic construct
  SITE 1: note = P is dP
  SITE 2: note = R is dR
  SITE 4: note = F is 4-CF3 modified F
  SITE 7: note = T is dT
PRRFKRT

SEQ ID NO: 14 - protein, 5 aa, synthetic construct
  SITE 2: note = A is 4-Pip modified A
RAKRT

SEQ ID NO: 15 - protein, 5 aa, synthetic construct
  SITE 2: note = A is 4-Pip modified A
  SITE 5: note = T is dT
RAKRT

SEQ ID NO: 16 - protein, 6 aa, synthetic construct
  SITE 3: note = A is 4-Pip modified A
  SITE 6: note = T is dT
RRAKRT

SEQ ID NO: 17 - protein, 6 aa, synthetic construct
  SITE 1: note = R is dR
  SITE 3: note = A is 4-Pip modified A
  SITE 6: note = T is dT
RRAKRT

SEQ ID NO: 18 - protein, 7 aa, synthetic construct
  SITE 2: note = R is dR
  SITE 4: note = A is 4-Pip modified A
  SITE 7: note = T is dT
PRRAKRT

SEQ ID NO: 19 - protein, 7 aa, synthetic construct
  SITE 1: note = P is dP
  SITE 2: note = R is dR
  SITE 4: note = A is 4-Pip modified A
  SITE 7: note = T is dT
PRRAKRT

SEQ ID NO: 20 - protein, 5 aa, synthetic construct
  SITE 2: note = F is 4-Guan modified F
RFKRT

SEQ ID NO: 21 - protein, 5 aa, synthetic construct
  SITE 2: note = F is 4-Guan modified F
  SITE 5: note = T is dT
RFKRT

SEQ ID NO: 22 - protein, 6 aa, synthetic construct
  SITE 3: note = F is 4-Guan modified F
  SITE 6: note = T is dT
RRFKRT

SEQ ID NO: 23 - protein, 6 aa, synthetic construct
  SITE 1: note = R is dR
  SITE 3: note = F is 4-Guan modified F
  SITE 6: note = T is dT
RRFKRT

SEQ ID NO: 24 - protein, 7 aa, synthetic construct
  SITE 2: note = R is dR
  SITE 4: note = F is 4-Guan modified F
  SITE 7: note = T is dT
PRRFKRT

SEQ ID NO: 25 - protein, 7 aa, synthetic construct
  SITE 1: note = P is dP
  SITE 2: note = R is dR
  SITE 4: note = F is 4-Guan modified F
  SITE 7: note = T is dT
PRRFKRT